European Patent Specification EP 4 038 180 B1, published January 3, 2024. Title: Treatment of Chronic Granulomatous Disease. Applicant: Universität Zürich. The sequence listing filed with the application follows.

SEQUENCE LISTING (2 sequences)

SEQ ID NO: 1 - DNA, 778 bp, Homo sapiens
acttgtacagcttcacagggctccatgcttagaaggaccccacacttagtttaatgttctgctgtcatcatcttgatattcttaatttttaaataaagggcctatcgttttcattttttactgggccttgcaaattatgtagctggttctgtatgccaggagagaagttggaagtaaaatggtattccaggaccaggaggcattctggcagagtgaaagaacatgtgatttggagtccatggggatgggtttaaatttcagctttccactaatttgctttgtgatactgagtatttccttttatccctcagaggctctgtttctcaattttgactacgggttttttcattagataatgtctcagttctggtattccaggtttccctcaattattctgggaaaacctccttgacccacaggcagagcctagggcagccaggtgctttctactctctctctctctgcagcttggaaagttagtgtctgttgaaggtcagctgggagttggtggaggcagggcagtggcctgctactattgctgcagtagcagaccctttcacaacagcattgttttgtcattttgcatccagatttccgttggctaacctcagtcttatcttcctcatttctgtttcctgttgaagacaccaagggcccttcaaaacacagaagcttcttgctcacggcagaaagcccaattccatctggcccctgcaggttggctcagcactggggaatcagagtcccctccatgaccaaggcaccactccactgacag

SEQ ID NO: 2 - DNA, 8688 bp, Homo sapiens
ccattgcatacgttgtatccatatcataatatgtacatttatattggctcatgtccaacattaccgccatgttgacattgattattgactagttattaatagtaatcaattacggggtcattagttcatagcccatatatggagttccgcgttacataacttacggtaaatggcccgcctggctgaccgcccaacgacccccgcccattgacgtcaataatgacgtatgttcccatagtaacgccaatagggactttccattgacgtcaatgggtggagtatttacggtaaactgcccacttggcagtacatcaagtgtatcatatgccaagtacgccccctattgacgtcaatgacggtaaatggcccgcctggcattatgcccagtacatgaccttatgggactttcctacttggcagtacatctacgtattagtcatcgctattaccatggtgatgcggttttggcagtacatcaatgggcgtggatagcggtttgactcacggggatttccaagtctccaccccattgacgtcaatgggagtttgttttggcaccaaaatcaacgggactttccaaaatgtcgtaacaactccgccccattgacgcaaatgggcggtaggcgtgtacggtgggaggtctatataagcagagctcgtttagtgaaccggggtctctctggttagaccagatctgagcctgggagctctctggctaactagggaacccactgcttaagcctcaataaagcttgccttgagtgcttcaagtagtgtgtgcccgtctgttgtgtgactctggtaactagagatccctcagacccttttagtcagtgtggaaaatctctagcagtggcgcccgaacagggacttgaaagcgaaagggaaaccagaggagctctctcgacgcaggactcggcttgctgaagcgcgcacggcaagaggcgaggggcggcgactggtgagtacgccaaaaattttgactagcggaggctagaaggagagagatgggtgcgagagcgtcagtattaagcgggggagaattagatcgcgatgggaaaaaattcggttaaggccagggggaaagaaaaaatataaattaaaacatatagtatgggcaagcagggagctagaacgattcgcagttaatcctggcctgttagaaacatcagaaggctgtagacaaatactgggacagctacaaccatcccttcagacaggatcagaagaacttagatcattatataatacagtagcaaccctctattgtgtgcatcaaaggatagagataaaagacaccaaggaagctttagacaagatagaggaagagcaaaacaaaagtaagaccaccgcacagcaagcggccgctgatcttcagacctggaggaggagatatgagggacaattggagaagtgaattatataaatataaagtagtaaaaattgaaccattaggagtagcacccaccaaggcaaagagaagagtggtgcagagagaaaaaagagcagtgggaataggagctttgttccttgggttcttgggagcagcaggaagcactatgggcgcagcgtcaatgacgctgacggtacaggccagacaattattgtctggtatagtgcagcagcagaacaatttgctgagggctattgaggcgcaacagcatctgttgcaactcacagtctggggcatcaagcagctccaggcaagaatcctggctgtggaaagatacctaaaggatcaacagctcctggggatttggggttgctctggaaaactcatttgcaccactgctgtgccttggaatgctagttggagtaataaatctctggaacagatttggaatcacacgacctggatggagtgggacagagaaattaacaattacacaagcttaatacactccttaattgaagaatcgcaaaaccagcaagaaaagaatgaacaagaattattggaattagataaatgggcaagtttgtggaattggtttaacataacaaattggctgtggtatataaaattattcataatgatagtaggaggcttggtaggtttaagaatagtttttgctgtactttctatagtgaatagagttaggcagggatattcaccattatcgtttcagacccacctcccaaccccgaggggacccgacaggcccgaaggaatagaagaagaaggtggagagagagacagagacagatccattcgattagtgaacggatctcgacggtatcggttaacttttaaaagaaaaggggggattggggggtacagtgcaggggaaagaatagtagacataatagcaacagacatacaaactaaagaattacaaaaacaaattacaaaaattcaaaattttatcgatcacgagactagcctcgagaagcttgatataatagtcgacacttgtacagcttcacagggctccatgcttagaaggaccccacacttagtttaatgttctgctgtcatcatcttgatattcttaatttttaaataaagggcctatcgttttcattttttactgggccttgcaaattatgtagctggttctgtatgccaggagagaagttggaagtaaaatggtattccaggaccaggaggcattctggcagagtgaaagaacatgtgatttggagtccatggggatgggtttaaatttcagctttccactaatttgctttgtgatactgagtatttccttttatccctcagaggctctgtttctcaattttgactacgggttttttcattagataatgtctcagttctggtattccaggtttccctcaattattctgggaaaacctccttgacccacaggcagagcctagggcagccaggtgctttctactctctctctctctgcagcttggaaagttagtgtctgttgaaggtcagctgggagttggtggaggcagggcagtggcctgctactattgctgcagtagcagaccctttcacaacagcattgttttgtcattttgcatccagatttccgttggctaacctcagtcttatcttcctcatttctgtttcctgttgaagacaccaagggcccttcaaaacacagaagcttcttgctcacggcagaaagcccaattccatctggcccctgcaggttggctcagcactggggaatcagagtcccctccatgaccaaggcaccactccactgacagggatccaagcttgccaccatgggcgacaccttcatccggcacatcgccctgctgggcttcgagaagcggttcgtgcccagccagcactacgtgtacatgtttctggtgaagtggcaggacctgagcgagaaggtggtgtaccggcggttcaccgagatctacgagttccacaagaccctgaaagagatgttccccatcgaggccggagccatcaaccccgagaaccggatcatcccccacctgcctgcccccaagtggttcgacggccagagagccgccgagaacaggcagggcaccctgaccgagtactgcagcaccctgatgagcctgcccaccaagatcagccggtgccctcacctgctggatttcttcaaagtgcggcccgacgacctgaagctgcccaccgacaaccagaccaagaagcccgagacctacctgatgcccaaggacggcaagagcaccgccaccgacatcaccggccccatcatcctgcagacctaccgggccatcgccgactacgagaaaaccagcggcagcgagatggccctgagcaccggcgacgtggtggaggtggtggaaaagagcgagagcgggtggtggttctgccagatgaaggccaagcggggctggattcccgccagcttcctggaacccctggacagccccgacgagaccgaggaccccgagcccaactacgccggcgagccctacgtggccatcaaggcctacaccgccgtggagggcgacgaggtgtccctgctggaaggcgaggccgtggaggtgatccacaagctgctggacggatggtgggtgatccggaaggacgacgtgaccggctacttccccagcatgtacctgcagaagagcggccaggacgtcagccaggcccagcggcagatcaagagaggcgcccctcccaggcggagcagcatccggaacgcccacagcatccaccagagaagccggaagagactgagccaggacgcctaccggcggaacagcgtgcggttcctgcagcagcggcggaggcaggccagacccggccctcagagccccggcagccccctggaagaggaacggcagacccagcggagcaagccccagcccgccgtgccccctagacccagcgccgacctgatcctgaaccggtgcagcgagagcaccaagcggaagctggccagcgccgtgtgatgactcgagtattatatcaagcttatcgataccgtcgaatcccccgggctgcaggaattcgagcatcttaccgccatttattcccatatttgttctgtttttcttgatttgggtatacatttaaatgttaataaaacaaaatggtggggcaatcatttacatttttagggatatgtaattactagttcaggtgtattgccacaagacaaacatgttaagaaactttcccgttatttacgctctgttcctgttaatcaacctctggattacaaaatttgtgaaagattgactgatattcttaactatgttgctccttttacgctgtgtggatatgctgctttaatgcctctgtatcatgctattgcttcccgtacggctttcgttttctcctccttgtataaatcctggttgctgtctctttatgaggagttgtggcccgttgtccgtcaacgtggcgtggtgtgctctgtgtttgctgacgcaacccccactggctggggcattgccaccacctgtcaactcctttctgggactttcgctttccccctcccgatcgccacggcagaactcatcgccgcctgccttgcccgctgctggacaggggctaggttgctgggcactgataattccgtggtgttgtcggggaagggcctgctgccggctctgcggcctcttccgcgtcttcgccttcgccctcagacgagtcggatctccctttgggccgcctccccgcctggaattcgagctcggtacctttaagaccaatgacttacaaggcagctgtagatcttagccactttttaaaagaaaaggggggactggaagggctaattcactcccaacgaagacaagatctgctttttgcttgtactgggtctctctggttagaccagatctgagcctgggagctctctggctaactagggaacctactgcttaagcctcaataaagcttgccttgagtgcttcaagtagtgtgtgcccgtctgttgtgtgactctggtaactagagatccctcagacccttttagtcagtgtggaaaatctctagcagtagtagttcatgtcatcttattattcagtatttataacttgcaaagaaatgaatatcagagagtgagaggaacttgtttattgcagcttataatggttacaaataaagcaatagcatcacaaatttcacaaataaagcatttttttcactgcattctagttgtggtttgtccaaactcatcaatgtatcttatcatgtctggctctagctatcccgcccctaactccgcccatcccgcccctaactccgcccagttccgcccattctccgccccatggctgactaattttttttatttatgcagaggccgaggccgcctcggcctctgagctattccagaagtagtgaggaggcttttttggaggcctagggacgtacccaattcgccctatagtgagtcgtattacgcgcgctcactggccgtcgttttacaacgtcgtgactgggaaaaccctggcgttacccaacttaatcgccttgcagcacatccccctttcgccagctggcgtaatagcgaagaggcccgcaccgatcgcccttcccaacagttgcgcagcctgaatggcgaatgggacgcgccctgtagcggcgcattaagcgcggcgggtgtggtggttacgcgcagcgtgaccgctacacttgccagcgccctagcgcccgctcctttcgctttcttcccttcctttctcgccacgttcgccggctttccccgtcaagctctaaatcgggggctccctttagggttccgatttagtgctttacggcacctcgaccccaaaaaacttgattagggtgatggttcacgtagtgggccatcgccctgatagacggtttttcgccctttgacgttggagtccacgttctttaatagtggactcttgttccaaactggaacaacactcaaccctatctcggtctattcttttgatttataagggattttgccgatttcggcctattggttaaaaaatgagctgatttaacaaaaatttaacgcgaattttaacaaaatattaacgcttacaatttaggtggcacttttcggggaaatgtgcgcggaacccctatttgtttatttttctaaatacattcaaatatgtatccgctcatgagacaataaccctgataaatgcttcaataatagcacctagatcaagagacaggatgaggatcgtttcgcatgattgaacaagatggattgcacgcaggttctccggccgcttgggtggagaggctattcggctatgactgggcacaacagacaatcggctgctctgatgccgccgtgttccggctgtcagcgcaggggcgcccggttctttttgtcaagaccgacctgtccggtgccctgaatgaactgcaagacgaggcagcgcggctatcgtggctggccacgacgggcgttccttgcgcagctgtgctcgacgttgtcactgaagcgggaagggactggctgctattgggcgaagtgccggggcaggatctcctgtcatctcaccttgctcctgccgagaaagtatccatcatggctgatgcaatgcggcggctgcatacgcttgatccggctacctgcccattcgaccaccaagcgaaacatcgcatcgagcgagcacgtactcggatggaagccggtcttgtcgatcaggatgatctggacgaagagcatcaggggctcgcgccagccgaactgttcgccaggctcaaggcgagcatgcccgacggcgaggatctcgtcgtgacccatggcgatgcctgcttgccgaatatcatggtggaaaatggccgcttttctggattcatcgactgtggccggctgggtgtggcggaccgctatcaggacatagcgttggctacccgtgatattgctgaagagcttggcggcgaatgggctgaccgcttcctcgtgctttacggtatcgccgctcccgattcgcagcgcatcgccttctatcgccttcttgacgagttcttctgaattattaacgcttacaatttcctgatgcggtattttctccttacgcatctgtgcggtatttcacaccgcatcaggtggcacttttcggggaaatgtgcgcggaacccctatttgtttatttttctaaatacattcaaatatgtatccgctcatgaccaaaatcccttaacgtgagttttcgttccactgagcgtcagaccccgtagaaaagatcaaaggatcttcttgagatcctttttttctgcgcgtaatctgctgcttgcaaacaaaaaaaccaccgctaccagcggtggtttgtttgccggatcaagagctaccaactctttttccgaaggtaactggcttcagcagagcgcagataccaaatactgttcttctagtgtagccgtagttaggccaccacttcaagaactctgtagcaccgcctacatacctcgctctgctaatcctgttaccagtggctgctgccagtggcgataagtcgtgtcttaccgggttggactcaagacgatagttaccggataaggcgcagcggtcgggctgaacggggggttcgtgcacacagcccagcttggagcgaacgacctacaccgaactgagatacctacagcgtgagctatgagaaagcgccacgcttcccgaagggagaaaggcggacaggtatccggtaagcggcagggtcggaacaggagagcgcacgagggagcttccagggggaaacgcctggtatctttatagtcctgtcgggtttcgccacctctgacttgagcgtcgatttttgtgatgctcgtcaggggggcggagcctatggaaaaacgccagcaacgcggcctttttacggttcctggccttttgctggccttttgctcacatgttctttcctgcgttatcccctgattctgtggataaccgtattaccgcctttgagtgagctgataccgctcgccgcagccgaacgaccgagcgcagcgagtcagtgagcgaggaagcggaagagcgcccaatacgcaaaccgcctctccccgcgcgttggccgattcattaatgcagctggcacgacaggtttcccgactggaaagcgggcagtgagcgcaacgcaattaatgtgagttagctcactcattaggcaccccaggctttacactttatgcttccggctcgtatgttgtgtggaattgtgagcggataacaatttcacacaggaaacagctatgaccatgattacgccaagcgcgcaattaaccctcactaaagggaacaaaagctggagctgcaagcttgg